European Patent Application EP 4 793 352 A1, published August 19, 2026. Title: GENOME EDITING METHOD AND METHOD FOR PRODUCING GENOME-EDITED PLANT. Applicant: KANEKA CORPORATION. The sequence listing filed with the application follows.

SEQUENCE LISTING (13 sequences)

SEQ ID NO: 1 - RNA, 42 nt, synthetic construct
  source 1..42: mol_type = other RNA
acccaagtaaagtaccaagggttttagagctatgctgttttg

SEQ ID NO: 2 - RNA, 69 nt, synthetic construct
  source 1..69: mol_type = other RNA
aaacagcatagcaagttaaaataaggctagtccgttatcaacttgaaaaagtggcaccgagtcggtgct

SEQ ID NO: 3 - DNA, 24 bp, synthetic construct
  source 1..24: mol_type = other DNA
atgtgtcgcagcaaatcaaaatgg

SEQ ID NO: 4 - DNA, 20 bp, synthetic construct
  source 1..20: mol_type = other DNA
acgcccaaccgcttcctata

SEQ ID NO: 5 - DNA, 20 bp, synthetic construct
  source 1..20: mol_type = other DNA
atttggaaacggcagagaag

SEQ ID NO: 6 - DNA, 19 bp, synthetic construct
  source 1..19: mol_type = other DNA
gagctcggtagcaattccc

SEQ ID NO: 7 - DNA, 38 bp, synthetic construct
  source 1..38: mol_type = other DNA
gtgctggaattcaggttgctgacatcactcctcaagag

SEQ ID NO: 8 - DNA, 38 bp, synthetic construct
  source 1..38: mol_type = other DNA
ctgccgtttccaaattggtactttacttgggtgatgac

SEQ ID NO: 9 - DNA, 38 bp, synthetic construct
  source 1..38: mol_type = other DNA
attgctaccgagctcagggggctgtggtatgtgaaacc

SEQ ID NO: 10 - DNA, 37 bp, synthetic construct
  source 1..37: mol_type = other DNA
tctgcagaattcaggtatcacatttaacttttcaacg

SEQ ID NO: 11 - DNA, 16 bp, synthetic construct
  source 1..16: mol_type = other DNA
gtaaaacgacggccag

SEQ ID NO: 12 - DNA, 17 bp, synthetic construct
  source 1..17: mol_type = other DNA
caggaaacagctatgac

SEQ ID NO: 13 - RNA, 20 nt, synthetic construct
  source 1..20: mol_type = other RNA
tgagccagatgcgctcctcg